European Patent Application EP 4 574 956 A1, published June 25, 2025. Title: LIQUID DETERGENT COMPOSITIONS. Applicant: The Procter & Gamble Company. The sequence listing filed with the application follows.

SEQUENCE LISTING (8 sequences)

SEQ ID NO: 1 - protein, 773 aa, Halalkalibacter akibai
AEGNTREDNFKHLLGNDNVKRPSEAGALQLQEVDGQMTLVDQHGEKIQLRGMSTHGLQWFPEILNDNAYKALANDWESNMIRLAMYVGENGYASNPELIKSRVIKGIDLAIENDMYVIVDWHVHAPGDPRDPVYAGAEDFFRDIAALYPNNPHIIYELANEPSSNNNGGAGIPNNEEGWNAVKEYADPIVEMLRDSGNADDNIIIVGSPNWSQRPDLAADNPINDHHTMYTVHFYTGSHAASTESYPPETPNSERGNVMSNTRYALENGVAVFATEWGTSQANGDGGPYFDEADVWIEFLNENNISWANWSLTNKNEVSGAFTPFELGKSNATNLDPGPDHVWAPEELSLSGEYVRARIKGVNYEPIDRTKYTKVLWDFNDGTKQGFGVNSDSPNKELIAVDNENNTLKVSGLDVSNDVSDGNFWANARLSADGWGKSVDILGAEKLTMDVIVDEPTTVAIAAIPQSSKSGWANPERAVRVNAEDFVQQTDGKYKAGLTITGEDAPNLKNIAFHEEDNNMNNIILFVGTDAADVIYLDNIKVIGTEVEIPVVHDPKGEAVLPSVFEDGTRQGWDWAGESGVKTALTIEEANGSNALSWEFGYPEVKPSDNWATAPRLDFWKSDLVRGENDYVAFDFYLDPVRATEGAMNINLVFQPPTNGYWVQAPKTYTINFDELEEANQVNGLYHYEVKINVRDITNIQDDTLLRNMMIIFADVESDFAGRVFVDNVRFEGAATTEPVEPEPVDPGEETPPVDEKEAKKEQKEAEKEEKEE

SEQ ID NO: 2 - protein, 294 aa, Sordaria fimicola
MRSSTILQTGLVAVLPFAVQAASGSGKSTRYWDCCKPSCAWSGKASVNRPVLACDANNNPLNDANVKSGCDGGSAYTCANNSPWAVNDNLAYGFAATKLSGGTESSWCCACYALTFTSGPVSGKTLVVQSTSTGGDLGSNHFDLNMPGGGVGLFDGCKREFGGLPGAQYGGISSRSECDSFPAALKPGCQWRFDWFKNADNPEFTFKQVQCPSELTSRTGCKRNDDSQFPAFTPPSGGGSNPSTPTTPPSSGGGGSGCAAAMYAQCGGSGFSGCTNCPSGSTCKAINDYYHQCA

SEQ ID NO: 3 - protein, 305 aa, Humicola insolens
MRSSPLLRSAVVAALPVLALAADGRSTRYWDCCKPSCGWAKKAPVNQPVFSCNANFQRITDFDAKSGCEPGGVAYSCADQTPWAVNDDFALGFAATSIAGSNEAGWCCACYELTFTSGPVAGKKMVVQSTSTGGDLGSNHFDLNIPGGGVGIFDGCTPQFGGLPGQRYGGISSRNECDRFPDALKPGCYWRFDWFKNADNPSFSFRQVQCPAELVARTGCRRNDDGNFPAVQIPSSSTSSPVNQPTSTSTTSTSTTSSPPVQPTTPSGCTAERWAQCGGNGWSGCTTCVAGSTCTKINDWYHQCL

SEQ ID NO: 4 - protein, 299 aa, Thielavia terrestris
MRSTPVLRTTLAAALPLVASAASGSGQSTRYWDCCKPSCAWPGKAAVSQPVYACDANFQRLSDFNVQSGCNGGSAYSCADQTPWAVNDNLAYGFAATSIAGGSESSWCCACYALTFTSGPVAGKTMVVQSTSTGGDLGSNHFDIAMPGGGVGIFNGCSSQFGGLPGAQYGGISSRDQCDSFPAPLKPGCQWRFDWFQNADNPTFTFQQVQCPAEIVARSGCKRNDDSSFPVFTPPSGGNGGTGTPTSTAPGSGQTSPGGGSGCTSQKWAQCGGIGFSGCTTCVSGTTCQKLNDYYSQCL

SEQ ID NO: 5 - protein, 295 aa, Staphylotrichum coccosporum
ADGKSTRYWDCCKPSCSWPGKASVNQPVFACSANFQRISDPNVKSGCDGGSAYACADQTPWAVNDNFSYGFAATSISGGNEASWCCGCYELTFTSGPVAGKTMVVQSTSTGGDLGTNHFDLAMPGGGVGIFDGCSPQFGGLAGDRYGGVSSRSQCDSFPAALKPGCYWRFDWFKNADNPTFTFRQVQCPSELVARTGCRRNDDGNFPVFTPPSGGQSSSSSSSSSAKPTSTSTSTTSTKATSTTSTASSQTSSSTGGGCAAQRWAQCGGIGFSGCTTCVSGTTCNKQNDWYSQCL

SEQ ID NO: 6 - protein, 214 aa, Melanocarpus albomyces
ANGQSTRYWDCCKPSCGWRGKGPVNQPVYSCDANFQRIHDFDAVSGCEGGPAFSCADHSPWAINDNLSYGFAATALSGQTEESWCCACYALTFTSGPVAGKTMVVQSTSTGGDLGSNHFDLNIPGGGVGLFDGCTPQFGGLPGARYGGISSRQECDSFPEPLKPGCQWRFDWFQNADNPSFTFERVQCPEELVARTGCRRHDDGGFAVFKAPSA

SEQ ID NO: 7 - protein, 524 aa, Paenibacillus polymyxa
VVHGQTAKTITIKVDTFKDRKPISPYIYGTNQDLAGDENMAARRLGGNRMTGYNWENNMSNAGSDWQQSSDNYLCSNGGLTQAECEKPGAVTTSFHDQSLKLGTYSLVTLPMAGYVAKDGNGSVQESEKAPSARWNQVVNAKNAPFQLQPDLNDNRVYVDEFVHFLVNKYGTASTKAGVKGYALDNEPALWSHTHPRIHGEKVGAKELVDRSVSLSKAVKAIDAGAEVFGPVLYGFGAYKDLQTAPDWDSVKGNYSWFVDYYLDQMRLSSQVEGKRLLDVFDVHWYPEAMGGGIRITNEVGNDETKKARMQAPRTLWDPTYKEDSWIAQWNSEFLPILPRLKQSVDKYYPGTKLAMTEYSYGGENDISGGIAMTDVLGILGKNDVYMANYWKLKDGVNNYVSAAYKLYRNYDGKNSTFGDTSVSAQTSDIVNSSVHASVTNASDKELHLVVMNKSMDSAFDAQFDLSGAKTYISGKVWGFDKNSSQIKEAAPITQISGNRFTYTVPPLTAYHIVLTTGNDTSPV

SEQ ID NO: 8 - protein, 415 aa, Humicola insolens
QKPGETKEVHPQLTTFRCTKRGGCKPATNFIVLDSLSHPIHRAEGLGPGGCGDWGNPPPKDVCPDVESCAKNCIMEGIPDYSQYGVTTNGTSLRLQHILPDGRVPSPRVYLLDKTKRRYEMLHLTGFEFTFDVDATKLPCGMNSALYLSEMHPTGAKSKYNSGGAYYGTGYCDAQCFVTPFINGLGNIEGKGSCCNEMDIWEVNSRASHVVPHTCNKKGLYLCEGEECAFEGVCDKNGCGWNNYRVNVTDYYGRGEEFKVNTLKPFTVVTQFLANRRGKLEKIHRFYVQDGKVIESFYTNKEGVPYTNMIDDEFCEATGSRKYMELGATQGMGEALTRGMVLAMSIWWDQGGNMEWLDHGEAGPCAKGEGAPSNIVQVEPFPEVTYTNLRWGEIGSTYQEVQKPKPKPGHGPRSD